European Patent Specification EP 3 543 258 B1, published September 13, 2023. Title: TEM-1 DIAGNOSTIC ANTIBODIES. Applicant: MORPHOTEK, INC. The sequence listing filed with the application follows.

SEQUENCE LISTING (161 sequences)

SEQ ID NO: 1 - protein, 11 aa, Artificial Sequence
  source: /note="Description of Artificial Sequence: Synthetic peptide"
QSLLDSDGNTY

SEQ ID NO: 2 - protein, 3 aa, Artificial Sequence
  source: /note="Description of Artificial Sequence: Synthetic peptide"
LVS

SEQ ID NO: 3 - protein, 9 aa, Artificial Sequence
  source: /note="Description of Artificial Sequence: Synthetic peptide"
MQATHAPFT

SEQ ID NO: 4 - protein, 131 aa, Artificial Sequence
  source: /note="Description of Artificial Sequence: Synthetic polypeptide"
MSPVQSLFLLLLWILGTKGDVVLTQTPSILSATIGQSVSISCRSSQSLLDSDGNTYLYWFLQRPGQSPQRLIYLVSNLGSGVPNRFSGSGSGTDFTLKISGVEAGDLGVYYCMQATHAPFTFGSGTKLEIK

SEQ ID NO: 5 - protein, 8 aa, Artificial Sequence
  source: /note="Description of Artificial Sequence: Synthetic peptide"
GFDFKTYA

SEQ ID NO: 6 - protein, 10 aa, Artificial Sequence
  source: /note="Description of Artificial Sequence: Synthetic peptide"
ISTKGHNYAT

SEQ ID NO: 7 - protein, 9 aa, Artificial Sequence
  source: /note="Description of Artificial Sequence: Synthetic peptide"
TVAGYNFDY

SEQ ID NO: 8 - protein, 136 aa, Artificial Sequence
  source: /note="Description of Artificial Sequence: Synthetic polypeptide"
MVLLELVSVIALFQGVHCEVQLVESGGGLVQPKGSLKLSCAASGFDFKTYAMSWVRQAPGKGLDWIVTISTKGHNYATLYADSVKERFTISRDDSQSMVYLQMNNLKTEDTALYYCTVAGYNFDYWGQGVMVTVSS

SEQ ID NO: 9 - protein, 6 aa, Artificial Sequence
  source: /note="Description of Artificial Sequence: Synthetic peptide"
QSVGIN

SEQ ID NO: 10 - protein, 3 aa, Artificial Sequence
  source: /note="Description of Artificial Sequence: Synthetic peptide"
TAS

SEQ ID NO: 11 - protein, 9 aa, Artificial Sequence
  source: /note="Description of Artificial Sequence: Synthetic peptide"
LQYGSLPFT

SEQ ID NO: 12 - protein, 127 aa, Artificial Sequence
  source: /note="Description of Artificial Sequence: Synthetic polypeptide"
MESHTRVFIFLLLWLSGGDGETVMTQSPTSMPTSIGERVTLNCKASQSVGINVDWYQQTPGQSPKLLIYTASNRHTGVPDRFAGSGSGRDFTLTISNVEAEDLVVYYCLQYGSLPFTFGAGTKLELK

SEQ ID NO: 13 - protein, 8 aa, Artificial Sequence
  source: /note="Description of Artificial Sequence: Synthetic peptide"
GFTFSNFD

SEQ ID NO: 14 - protein, 8 aa, Artificial Sequence
  source: /note="Description of Artificial Sequence: Synthetic peptide"
ITYDGSRT

SEQ ID NO: 15 - protein, 13 aa, Artificial Sequence
  source: /note="Description of Artificial Sequence: Synthetic peptide"
ARHGSSYYWFFDF

SEQ ID NO: 16 - protein, 139 aa, Artificial Sequence
  source: /note="Description of Artificial Sequence: Synthetic polypeptide"
MDIRLSLAFLVLFIKDVQCEVQLVESGGGLVQPGRSMILSCAASGFTFSNFDMAWVRQAPKMGLEWVATITYDGSRTNYRDSVKGRFTISRDSAKNTLYLQMDSLTSEDTATYYCARHGSSYYWFFDFWGPGTMVTVSS

SEQ ID NO: 17 - protein, 6 aa, Artificial Sequence
  source: /note="Description of Artificial Sequence: Synthetic peptide"
HSVGTN

SEQ ID NO: 18 - protein, 3 aa, Artificial Sequence
  source: /note="Description of Artificial Sequence: Synthetic peptide"
DAS

SEQ ID NO: 19 - protein, 9 aa, Artificial Sequence
  source: /note="Description of Artificial Sequence: Synthetic peptide"
QQTQSWPLT

SEQ ID NO: 20 - protein, 127 aa, Artificial Sequence
  source: /note="Description of Artificial Sequence: Synthetic polypeptide"
MVFKFQILGLLLFWISASRGDIVLTQSPTTLSVTPGETVSLSCRASHSVGTNLHWYQQKTNESPRLLIKDASQSMSGIPSRFSASGSGTDFTLNIKNVEFDDVSSYFCQQTQSWPLTFGSGTKLEIK

SEQ ID NO: 21 - protein, 8 aa, Artificial Sequence
  source: /note="Description of Artificial Sequence: Synthetic peptide"
GFTFRNYY

SEQ ID NO: 22 - protein, 8 aa, Artificial Sequence
  source: /note="Description of Artificial Sequence: Synthetic peptide"
TGSGGDFT

SEQ ID NO: 23 - protein, 9 aa, Artificial Sequence
  source: /note="Description of Artificial Sequence: Synthetic peptide"
ARAYGYFDY

SEQ ID NO: 24 - protein, 135 aa, Artificial Sequence
  source: /note="Description of Artificial Sequence: Synthetic polypeptide"
MDIRLSLAFLVLFIEDVQCEVQLVESGGGLVQPGRSMKLSCAASGFTFRNYYMAWVRQAPTRGLEWVASTGSGGDFTYYRDSVKGRFTISRDTAENTLYLQMDSLRSEDTATYYCARAYGYFDYWGQGVRVTVSS

SEQ ID NO: 25 - protein, 12 aa, Artificial Sequence
  source: /note="Description of Artificial Sequence: Synthetic peptide"
QSLLYNENNKNY

SEQ ID NO: 26 - protein, 3 aa, Artificial Sequence
  source: /note="Description of Artificial Sequence: Synthetic peptide"
WAS

SEQ ID NO: 27 - protein, 9 aa, Artificial Sequence
  source: /note="Description of Artificial Sequence: Synthetic peptide"
QQYFRFPRT

SEQ ID NO: 28 - protein, 133 aa, Artificial Sequence
  source: /note="Description of Artificial Sequence: Synthetic polypeptide"
MESQTQVLMSLLLWVAGSCGDIVMTQTPSSQAVSAGEKVTMSCTSGQSLLYNENNKNYLAWYQLKPGQSPRLLIYWASTRESGVPDRFIGSGSGTYFTLTISSVQAEDLAVYYCQQYFRFPRTFGGGTKLELK

SEQ ID NO: 29 - protein, 8 aa, Artificial Sequence
  source: /note="Description of Artificial Sequence: Synthetic peptide"
GFSLTNYN

SEQ ID NO: 30 - protein, 7 aa, Artificial Sequence
  source: /note="Description of Artificial Sequence: Synthetic peptide"
IWSGGSA

SEQ ID NO: 31 - protein, 12 aa, Artificial Sequence
  source: /note="Description of Artificial Sequence: Synthetic peptide"
TRDQLGGWYFDF

SEQ ID NO: 32 - protein, 137 aa, Artificial Sequence
  source: /note="Description of Artificial Sequence: Synthetic polypeptide"
MAVLGLLLCLVTFPSCALSQVQLKESGPGLVQPSQTLSLTCTVSGFSLTNYNIHWVRQPPGKGLEWMGAIWSGGSADYDSALKSRLSISRDTSKSQVFLKMDNLQTEDTAIYYCTRDQLGGWYFDFWGPGTKVTVSS

SEQ ID NO: 33 - protein, 11 aa, Artificial Sequence
  source: /note="Description of Artificial Sequence: Synthetic peptide"
KSLLSIEGINS

SEQ ID NO: 34 - protein, 3 aa, Artificial Sequence
  source: /note="Description of Artificial Sequence: Synthetic peptide"
RMS

SEQ ID NO: 35 - protein, 9 aa, Artificial Sequence
  source: /note="Description of Artificial Sequence: Synthetic peptide"
AQFLEFPFT

SEQ ID NO: 36 - protein, 132 aa, Artificial Sequence
  source: /note="Description of Artificial Sequence: Synthetic polypeptide"
MKFPAQFLGLMVLCFPGATGDNVLTQAPLAVSVTPGESASISCRSSKSLLSIEGINSLYWYLQKPGKSPQLLLFRMSNLASGVPDRFSGSGSETDFTLKISQVETEDVGVYYCAQFLEFPFTFGSGTKLEIK

SEQ ID NO: 37 - protein, 8 aa, Artificial Sequence
  source: /note="Description of Artificial Sequence: Synthetic peptide"
GFSFSDYY

SEQ ID NO: 38 - protein, 8 aa, Artificial Sequence
  source: /note="Description of Artificial Sequence: Synthetic peptide"
ISYDGSGS

SEQ ID NO: 39 - protein, 8 aa, Artificial Sequence
  source: /note="Description of Artificial Sequence: Synthetic peptide"
ARGGGLDY

SEQ ID NO: 40 - protein, 134 aa, Artificial Sequence
  source: /note="Description of Artificial Sequence: Synthetic polypeptide"
MDIRLSLVFLVLFIKGVQCEVQLVESDGGLVQPGRSLKLSCAASGFSFSDYYMAWVRQAPTKGLEWVATISYDGSGSYYRDSVKGRFTVSRDNAKTTLYLQMDSLRSEDTATYYCARGGGLDYWGQGVMVTVSS

SEQ ID NO: 41 - protein, 12 aa, Artificial Sequence
  source: /note="Description of Artificial Sequence: Synthetic peptide"
QSLLYNKNKKNY

SEQ ID NO: 42 - protein, 3 aa, Artificial Sequence
  source: /note="Description of Artificial Sequence: Synthetic peptide"
WAS

SEQ ID NO: 43 - protein, 8 aa, Artificial Sequence
  source: /note="Description of Artificial Sequence: Synthetic peptide"
QQYYTFPT

SEQ ID NO: 44 - protein, 132 aa, Artificial Sequence
  source: /note="Description of Artificial Sequence: Synthetic polypeptide"
MESQTQVLMSLLLWVSGTCGDIVMTQTPSSQAVSAGAKVTLSCKSSQSLLYNKNKKNYLAWYQQKPGQSPKLLIYWASTRESGVPDRFIGSGSGTDFTLTISSVQAEDLAIYYCQQYYTFPTFGAGTKLELK

SEQ ID NO: 45 - protein, 8 aa, Artificial Sequence
  source: /note="Description of Artificial Sequence: Synthetic peptide"
GFTFSDYN

SEQ ID NO: 46 - protein, 8 aa, Artificial Sequence
  source: /note="Description of Artificial Sequence: Synthetic peptide"
ISYNGSEI

SEQ ID NO: 47 - protein, 18 aa, Artificial Sequence
  source: /note="Description of Artificial Sequence: Synthetic peptide"
ARHWREYYSSYSSYVMDA

SEQ ID NO: 48 - protein, 144 aa, Artificial Sequence
  source: /note="Description of Artificial Sequence: Synthetic polypeptide"
MDIRLSLVFLVLFMKGVQCEVQLVEFGGGLVQPGRSLKLSCAASGFTFSDYNLAWVRQAPKKGLEWVATISYNGSEIYYRDSVKGRFTISRDNAKNTLYLQMDSLRSEDTATYYCARHWREYYSSYSSYVMDAWGQGASVTVSS

SEQ ID NO: 49 - protein, 11 aa, Artificial Sequence
  source: /note="Description of Artificial Sequence: Synthetic peptide"
KSLLGSKGINF

SEQ ID NO: 50 - protein, 3 aa, Artificial Sequence
  source: /note="Description of Artificial Sequence: Synthetic peptide"
RMS

SEQ ID NO: 51 - protein, 9 aa, Artificial Sequence
  source: /note="Description of Artificial Sequence: Synthetic peptide"
AQFLEYPNS

SEQ ID NO: 52 - protein, 132 aa, Artificial Sequence
  source: /note="Description of Artificial Sequence: Synthetic polypeptide"
MKFPAQFLGLIVLCIPGATGDIVLTQAPLSVSVTPGESASISCRSSKSLLGSKGINFLYWYLQKPGKSPQLLIYRMSNLASGVPDRFSGSGSETDFILKISKVETEDVGVYYCAQFLEYPNSFGAGTKLELK

SEQ ID NO: 53 - protein, 8 aa, Artificial Sequence
  source: /note="Description of Artificial Sequence: Synthetic peptide"
GFSLTNYN

SEQ ID NO: 54 - protein, 7 aa, Artificial Sequence
  source: /note="Description of Artificial Sequence: Synthetic peptide"
MWSGGNT

SEQ ID NO: 55 - protein, 13 aa, Artificial Sequence
  source: /note="Description of Artificial Sequence: Synthetic peptide"
ARDSGYGEGRLDY

SEQ ID NO: 56 - protein, 138 aa, Artificial Sequence
  source: /note="Description of Artificial Sequence: Synthetic polypeptide"
MAVRVLLLCLVTFPTCALSQVQLMESGPGLVQPSETLSLTCTVSGFSLTNYNIHWVRQPPGKGLEWMGLMWSGGNTDYNSALKSRLTISRDTSKNQVFLKMNSLQSEDTTTYYCARDSGYGEGRLDYWGQGVMVTVSS

SEQ ID NO: 57 - protein, 6 aa, Artificial Sequence
  source: /note="Description of Artificial Sequence: Synthetic peptide"
HSVGTN

SEQ ID NO: 58 - protein, 3 aa, Artificial Sequence
  source: /note="Description of Artificial Sequence: Synthetic peptide"
YVS

SEQ ID NO: 59 - protein, 9 aa, Artificial Sequence
  source: /note="Description of Artificial Sequence: Synthetic peptide"
QQTQSWPLT

SEQ ID NO: 60 - protein, 127 aa, Artificial Sequence
  source: /note="Description of Artificial Sequence: Synthetic polypeptide"
MVFKFQILGLLLFWISASRGDIVLTQSPTTLSVTPGETVSLSCRASHSVGTNLHWYQQKPNESPRLLIKYVSQSNSGIPSRFSASGSGTDFTLNIKNVEFNDVSSYFCQQTQSWPLTFGAGTKLEIK

SEQ ID NO: 61 - protein, 8 aa, Artificial Sequence
  source: /note="Description of Artificial Sequence: Synthetic peptide"
GFTFRNYY

SEQ ID NO: 62 - protein, 8 aa, Artificial Sequence
  source: /note="Description of Artificial Sequence: Synthetic peptide"
TGTGGDFT

SEQ ID NO: 63 - protein, 9 aa, Artificial Sequence
  source: /note="Description of Artificial Sequence: Synthetic peptide"
ARAYGYFDY

SEQ ID NO: 64 - protein, 135 aa, Artificial Sequence
  source: /note="Description of Artificial Sequence: Synthetic polypeptide"
MDIRLSLAFLVLFIKGVQCEVQLVESGGGLVQPGRSMKLSCSASGFTFRNYYMAWVRQAPTRGLEWVASTGTGGDFTYYRDSVKGRFTISRDTAENTLYLQMDSLRSEDTATYYCARAYGYFDYWGQGVKVTVSS

SEQ ID NO: 65 - protein, 6 aa, Artificial Sequence
  source: /note="Description of Artificial Sequence: Synthetic peptide"
HSVGTN

SEQ ID NO: 66 - protein, 3 aa, Artificial Sequence
  source: /note="Description of Artificial Sequence: Synthetic peptide"
YVS

SEQ ID NO: 67 - protein, 9 aa, Artificial Sequence
  source: /note="Description of Artificial Sequence: Synthetic peptide"
QQTQSWPLT

SEQ ID NO: 68 - protein, 127 aa, Artificial Sequence
  source: /note="Description of Artificial Sequence: Synthetic polypeptide"
MVFKFQILGLLLFWISASRGDIVLTQSPTTLSVTPGETVSLSCRASHSVGTNLHWYQQKTNESPRLLIKYVSQSNSGIPSRFSASGSGTDFTLNIKDVEFDDVSSYFCQQTQSWPLTFGSGTKLEIK

SEQ ID NO: 69 - protein, 8 aa, Artificial Sequence
  source: /note="Description of Artificial Sequence: Synthetic peptide"
GFIFRNYY

SEQ ID NO: 70 - protein, 8 aa, Artificial Sequence
  source: /note="Description of Artificial Sequence: Synthetic peptide"
TGTGGDFT

SEQ ID NO: 71 - protein, 9 aa, Artificial Sequence
  source: /note="Description of Artificial Sequence: Synthetic peptide"
ARAYGYFDY

SEQ ID NO: 72 - protein, 135 aa, Artificial Sequence
  source: /note="Description of Artificial Sequence: Synthetic polypeptide"
MDIRLSLAFLVLFIKGVQCEVQLVESGGGLVQPGRSMKLSCSASGFIFRNYYMAWVRQAPTKGLEWVASTGTGGDFTYYRDSVKGRFTISRDTAESTLYLQMDSLKSEDTATYYCARAYGYFDYWGQGVKVTVSS

SEQ ID NO: 73 - protein, 6 aa, Artificial Sequence
  source: /note="Description of Artificial Sequence: Synthetic peptide"
QNIYKY

SEQ ID NO: 74 - protein, 3 aa, Artificial Sequence
  source: /note="Description of Artificial Sequence: Synthetic peptide"
NIN

SEQ ID NO: 75 - protein, 8 aa, Artificial Sequence
  source: /note="Description of Artificial Sequence: Synthetic peptide"
YQYNSGRA

SEQ ID NO: 76 - protein, 125 aa, Artificial Sequence
  source: /note="Description of Artificial Sequence: Synthetic polypeptide"
MAPVQLLGLLLLCLRAMRCDIQMTQSPSLLSASEGDRVTLSCKASQNIYKYLNWYQQKLGEAPKLLIYNINNLQTGIPSRFSGSGSGTDFTLTISSLQPEDVATYYCYQYNSGRAFGGGTKLELK

SEQ ID NO: 77 - protein, 8 aa, Artificial Sequence
  source: /note="Description of Artificial Sequence: Synthetic peptide"
GFTFSDYW

SEQ ID NO: 78 - protein, 10 aa, Artificial Sequence
  source: /note="Description of Artificial Sequence: Synthetic peptide"
IRNKLNNYVT

SEQ ID NO: 79 - protein, 15 aa, Artificial Sequence
  source: /note="Description of Artificial Sequence: Synthetic peptide"
TRIQRVITTGEYFDY

SEQ ID NO: 80 - protein, 143 aa, Artificial Sequence
  source: /note="Description of Artificial Sequence: Synthetic polypeptide"
MDLRLTYVFIVAILKGVLCEVKLEESGGGLVQPGMSVKLSCATSGFTFSDYWMEWVRQAPGKGLEWVAEIRNKLNNYVTNYGKPVRGRFTISRDDSKSIVYLQVNSIRSEDTGIYYCTRIQRVITTGEYFDYWGQGVMVTVSS

SEQ ID NO: 81 - DNA, 33 bp, Artificial Sequence
  source: /note="Description of Artificial Sequence: Synthetic oligonucleotide"
cagagtctcttagatagtgatggaaacacctat

SEQ ID NO: 82 - DNA, 9 bp, Artificial Sequence
  source: /note="Description of Artificial Sequence: Synthetic oligonucleotide"
ttggtatcc

SEQ ID NO: 83 - DNA, 27 bp, Artificial Sequence
  source: /note="Description of Artificial Sequence: Synthetic oligonucleotide"
atgcaagctacccatgctccattcacg

SEQ ID NO: 84 - DNA, 393 bp, Artificial Sequence
  source: /note="Description of Artificial Sequence: Synthetic polynucleotide"
atgagtcctgtccagtccctgtttttattattgctttggattctgggaaccaaaggtgatgttgtgctgacccagactccatccatattgtctgctaccattggacaatcggtctccatctcttgcaggtcaagtcagagtctcttagatagtgatggaaacacctatttatattggttcctacagaggccaggccagtctccacagcgtctaatttatttggtatccaacctgggatctggggtccccaacaggttcagtggcagtgggtcaggaacagatttcacactcaaaatcagtggggtggaggctggagatttgggagtttattactgcatgcaagctacccatgctccattcacgttcggctcagggacgaagttggaaataaaa

SEQ ID NO: 85 - DNA, 24 bp, Artificial Sequence
  source: /note="Description of Artificial Sequence: Synthetic oligonucleotide"
ggatttgacttcaaaacttatgcc

SEQ ID NO: 86 - DNA, 30 bp, Artificial Sequence
  source: /note="Description of Artificial Sequence: Synthetic oligonucleotide"
ataagcactaagggtcataattatgcaaca

SEQ ID NO: 87 - DNA, 27 bp, Artificial Sequence
  source: /note="Description of Artificial Sequence: Synthetic oligonucleotide"
actgtggcagggtataattttgattac

SEQ ID NO: 88 - DNA, 408 bp, Artificial Sequence
  source: /note="Description of Artificial Sequence: Synthetic polynucleotide"
atggttctcctggagttggtttccgtgattgctctttttcaaggcgtgcattgtgaggtgcagcttgttgagtctggtggagggctggtgcagcctaaagggtcattgaaactctcatgtgcagcctctggatttgacttcaaaacttatgccatgagctgggtccgccaggctccaggaaagggtctggattggattgttaccataagcactaagggtcataattatgcaacactttatgctgactcagtgaaagagagattcaccatctccagagatgattcacaaagcatggtttacttgcaaatgaacaacttgaaaactgaggacacagccttgtattactgtactgtggcagggtataattttgattactggggccaaggagtcatggtcacagtctcctca

SEQ ID NO: 89 - DNA, 18 bp, Artificial Sequence
  source: /note="Description of Artificial Sequence: Synthetic oligonucleotide"
cagagcgtgggtattaat

SEQ ID NO: 90 - DNA, 9 bp, Artificial Sequence
  source: /note="Description of Artificial Sequence: Synthetic oligonucleotide"
acggcatcc

SEQ ID NO: 91 - DNA, 27 bp, Artificial Sequence
  source: /note="Description of Artificial Sequence: Synthetic oligonucleotide"
ctgcaatatggctcccttccgttcacg

SEQ ID NO: 92 - DNA, 381 bp, Artificial Sequence
  source: /note="Description of Artificial Sequence: Synthetic polynucleotide"
atggagtcacatactagggtcttcatattcctgctgctctggttgtctggaggtgatggggaaactgtgatgacccagtctcccacatccatgcccacatcaataggagagagggtcaccctgaactgcaaggccagtcagagcgtgggtattaatgtagactggtaccaacagacaccagggcagtctccgaaactgctgatatatacggcatccaaccggcacactggggtccctgatcgcttcgcaggcagtgggtctgggagagatttcactctcaccatcagcaacgtggaggctgaagacctggttgtttattactgtctgcaatatggctcccttccgttcacgtttggagctgggaccaagctggagctgaaa

SEQ ID NO: 93 - DNA, 24 bp, Artificial Sequence
  source: /note="Description of Artificial Sequence: Synthetic oligonucleotide"
ggattcactttcagtaactttgac

SEQ ID NO: 94 - DNA, 24 bp, Artificial Sequence
  source: /note="Description of Artificial Sequence: Synthetic oligonucleotide"
attacttatgatggcagtagaact

SEQ ID NO: 95 - DNA, 39 bp, Artificial Sequence
  source: /note="Description of Artificial Sequence: Synthetic oligonucleotide"
gcaagacatggaagctcctactactggttctttgacttc

SEQ ID NO: 96 - DNA, 417 bp, Artificial Sequence
  source: /note="Description of Artificial Sequence: Synthetic polynucleotide"
atggacatcaggctcagcttggctttccttgtccttttcataaaagatgtccagtgtgaggtgcagctggtggagtctgggggaggcttggtgcagcctggaaggtccatgatactctcctgtgcagcctcaggattcactttcagtaactttgacatggcctgggtccgccaggctccaaagatgggtctggagtgggtcgcaaccattacttatgatggcagtagaactaactatcgagactccgtgaagggccgattcactatctccagagatagtgcaaagaacaccctatacctgcaaatggacagtctgacgtctgaggacacggccacttattactgtgcaagacatggaagctcctactactggttctttgacttctggggcccaggaaccatggtcaccgtgtcctca

SEQ ID NO: 97 - DNA, 18 bp, Artificial Sequence
  source: /note="Description of Artificial Sequence: Synthetic oligonucleotide"
catagtgttggcacaaat

SEQ ID NO: 98 - DNA, 9 bp, Artificial Sequence
  source: /note="Description of Artificial Sequence: Synthetic oligonucleotide"
gatgcctca

SEQ ID NO: 99 - DNA, 27 bp, Artificial Sequence
  source: /note="Description of Artificial Sequence: Synthetic oligonucleotide"
caacagactcaaagttggcccctcacg

SEQ ID NO: 100 - DNA, 381 bp, Artificial Sequence
  source: /note="Description of Artificial Sequence: Synthetic polynucleotide"
atggtgttcaaatttcagatccttggacttctgcttttctggatttcagcctctagaggggacatcgtgttgactcagtctccaaccaccctgtctgtgactccaggagagacagtcagtctttcctgcagggctagtcatagtgttggcacaaatctacactggtatcagcaaaaaacaaatgagtccccaaggcttctcatcaaggatgcctcacagtccatgtccgggatcccctccaggttcagtgccagtggatcagggacagattttactctcaacatcaaaaatgtggagtttgatgatgtctcgagttatttttgtcaacagactcaaagttggcccctcacgttcggttctgggaccaagctggagatcaaa

SEQ ID NO: 101 - DNA, 24 bp, Artificial Sequence
  source: /note="Description of Artificial Sequence: Synthetic oligonucleotide"
ggattcactttcagaaactattac

SEQ ID NO: 102 - DNA, 24 bp, Artificial Sequence
  source: /note="Description of Artificial Sequence: Synthetic oligonucleotide"
actggtagtggtggtgatttcact

SEQ ID NO: 103 - DNA, 27 bp, Artificial Sequence
  source: /note="Description of Artificial Sequence: Synthetic oligonucleotide"
gcaagggcctatggatactttgattac

SEQ ID NO: 104 - DNA, 405 bp, Artificial Sequence
  source: /note="Description of Artificial Sequence: Synthetic polynucleotide"
atggacatcaggctcagtttggctttccttgtccttttcatagaagatgtccagtgtgaggtgcagctggtggagtctgggggaggcctagtgcagcctggaaggtccatgaaactctcctgtgcagcctcaggattcactttcagaaactattacatggcctgggtccgccaggctccaacgaggggtctggagtgggtcgcatccactggtagtggtggtgatttcacttactatcgagactccgtgaagggccgattcactatctccagagatactgcagaaaacaccctatacctacaaatggacagtctgaggtctgaggacacggccacgtattactgtgcaagggcctatggatactttgattactggggccaaggagtcagggtcacagtctcctca

SEQ ID NO: 105 - DNA, 36 bp, Artificial Sequence
  source: /note="Description of Artificial Sequence: Synthetic oligonucleotide"
cagagtcttttatacaatgaaaacaataagaactac

SEQ ID NO: 106 - DNA, 9 bp, Artificial Sequence
  source: /note="Description of Artificial Sequence: Synthetic oligonucleotide"
tgggcatcc

SEQ ID NO: 107 - DNA, 27 bp, Artificial Sequence
  source: /note="Description of Artificial Sequence: Synthetic oligonucleotide"
cagcaatattttaggtttcctcggacg

SEQ ID NO: 108 - DNA, 399 bp, Artificial Sequence
  source: /note="Description of Artificial Sequence: Synthetic polynucleotide"
atggaatcacagacacaggtcctcatgtccctgctgctctgggtagctggttcctgtggggacattgtgatgacccagactccatcctcccaggctgtgtcagcaggggagaaggtcactatgagctgcacgtccggtcagagtcttttatacaatgaaaacaataagaactacttggcctggtaccagctgaaaccggggcagtctcctagactgctgatctactgggcatccactagggaatctggggtccctgatcgcttcataggcagtggatctgggacgtatttcactctgaccatcagcagtgtgcaggcagaagacctggctgtttattactgccagcaatattttaggtttcctcggacgttcggtggaggcaccaagctggaattgaaa

SEQ ID NO: 109 - DNA, 24 bp, Artificial Sequence
  source: /note="Description of Artificial Sequence: Synthetic oligonucleotide"
ggattctcactaaccaactataat

SEQ ID NO: 110 - DNA, 21 bp, Artificial Sequence
  source: /note="Description of Artificial Sequence: Synthetic oligonucleotide"
atttggagtggtggaagtgca

SEQ ID NO: 111 - DNA, 36 bp, Artificial Sequence
  source: /note="Description of Artificial Sequence: Synthetic oligonucleotide"
accagagatcaactgggaggctggtactttgacttc

SEQ ID NO: 112 - DNA, 411 bp, Artificial Sequence
  source: /note="Description of Artificial Sequence: Synthetic polynucleotide"
atggctgtcctggggctgttgctctgcctggtgacatttccaagctgtgccctgtcccaggtgcagctgaaggagtcaggacctggtctggtgcagccctcacagaccctgtccctcacctgcactgtctctggattctcactaaccaactataatatacactgggttcgacagcctccaggaaagggtctggagtggatgggagcaatttggagtggtggaagtgcagattatgattcagctctcaaatcccgactgagcatcagcagggacacctccaagagccaagttttcttgaaaatggacaatctgcaaactgaagacacagccatttactactgtaccagagatcaactgggaggctggtactttgacttctggggcccaggaaccaaggtcaccgtgtcctca

SEQ ID NO: 113 - DNA, 33 bp, Artificial Sequence
  source: /note="Description of Artificial Sequence: Synthetic oligonucleotide"
aagagtctgctaagtattgagggcattaattcc

SEQ ID NO: 114 - DNA, 9 bp, Artificial Sequence
  source: /note="Description of Artificial Sequence: Synthetic oligonucleotide"
cggatgtcc

SEQ ID NO: 115 - DNA, 27 bp, Artificial Sequence
  source: /note="Description of Artificial Sequence: Synthetic oligonucleotide"
gcacagtttctagaatttccattcacg

SEQ ID NO: 116 - DNA, 396 bp, Artificial Sequence
  source: /note="Description of Artificial Sequence: Synthetic polynucleotide"
atgaagtttcctgctcagtttcttggactgatggtgctctgttttcctggagccactggggataatgtgttgactcaagctccactcgctgtttctgtcactcctggagagtcagcttccatctcctgcaggtctagtaagagtctgctaagtattgagggcattaattccttgtattggtaccttcagaagccaggaaagtctcctcagctcctgctttttcggatgtccaaccttgcctcaggagttccagacaggtttagtggcagtgggtcagaaacagattttacactgaaaatcagtcaggtggagactgaggatgttggcgtttattactgtgcacagtttctagaatttccattcacgttcggctcagggacgaagttggaaataaaa

SEQ ID NO: 117 - DNA, 24 bp, Artificial Sequence
  source: /note="Description of Artificial Sequence: Synthetic oligonucleotide"
ggattcagtttcagtgactattac

SEQ ID NO: 118 - DNA, 24 bp, Artificial Sequence
  source: /note="Description of Artificial Sequence: Synthetic oligonucleotide"
attagttatgatggtagtggtagt

SEQ ID NO: 119 - DNA, 24 bp, Artificial Sequence
  source: /note="Description of Artificial Sequence: Synthetic oligonucleotide"
gcaagagggggtggtcttgattac

SEQ ID NO: 120 - DNA, 402 bp, Artificial Sequence
  source: /note="Description of Artificial Sequence: Synthetic polynucleotide"
atggacatcaggctcagcttggttttccttgtccttttcataaaaggtgtccagtgtgaggtgcagctggtggagtctgatggaggcttagtgcagcctggaaggtccctaaaactctcctgtgcagcctcaggattcagtttcagtgactattacatggcctgggtccgccaggctccaacgaaggggctggagtgggtcgcaaccattagttatgatggtagtggtagttactatcgagactccgtgaagggccgattcactgtctccagagataatgcaaaaaccaccctatacctgcaaatggacagtctgaggtctgaggacacggccacttattactgtgcaagagggggtggtcttgattactggggccaaggagtcatggtcacagtctcctca

SEQ ID NO: 121 - DNA, 36 bp, Artificial Sequence
  source: /note="Description of Artificial Sequence: Synthetic oligonucleotide"
cagagtcttttatacaataaaaacaaaaagaactac

SEQ ID NO: 122 - DNA, 9 bp, Artificial Sequence
  source: /note="Description of Artificial Sequence: Synthetic oligonucleotide"
tgggcatcc

SEQ ID NO: 123 - DNA, 24 bp, Artificial Sequence
  source: /note="Description of Artificial Sequence: Synthetic oligonucleotide"
cagcagtactatacctttcccacc

SEQ ID NO: 124 - DNA, 396 bp, Artificial Sequence
  source: /note="Description of Artificial Sequence: Synthetic polynucleotide"
atggaatcacagacacaggtcctcatgtccctgctgctctgggtatctggtacctgtggggacattgtgatgacccagactccatcctcccaggctgtgtcagcaggggcgaaggtcactttgagctgcaagtccagtcagagtcttttatacaataaaaacaaaaagaactacttggcctggtaccagcagaaaccagggcagtctcctaaactgctgatctactgggcatccactagggaatctggggtccctgatcgcttcataggcagtggatctgggacagatttcactctgaccatcagcagtgtgcaggcagaagacctggctatttattactgccagcagtactatacctttcccacctttggggctgggaccaagctggaactgaaa

SEQ ID NO: 125 - DNA, 24 bp, Artificial Sequence
  source: /note="Description of Artificial Sequence: Synthetic oligonucleotide"
ggattcactttcagtgactataat

SEQ ID NO: 126 - DNA, 24 bp, Artificial Sequence
  source: /note="Description of Artificial Sequence: Synthetic oligonucleotide"
attagttataatggtagtgaaatt

SEQ ID NO: 127 - DNA, 54 bp, Artificial Sequence
  source: /note="Description of Artificial Sequence: Synthetic oligonucleotide"
gcaagacattggcgggaatactatagcagttattcctcctatgttatggatgcc

SEQ ID NO: 128 - DNA, 432 bp, Artificial Sequence
  source: /note="Description of Artificial Sequence: Synthetic polynucleotide"
atggacatcaggctcagcttggttttccttgtcctttttatgaaaggtgtccagtgtgaggtgcagctggtggagtttgggggaggcttagtgcagcctggaaggtccctgaaactctcctgtgcagcctcaggattcactttcagtgactataatttggcctgggtccgccaggctccaaagaagggtctggagtgggtcgcaaccattagttataatggtagtgaaatttactatcgagactccgtgaagggccgattcaccatctccagagataatgcaaaaaacaccctatatctgcagatggacagtctgaggtctgaggacacggccacttattactgtgcaagacattggcgggaatactatagcagttattcctcctatgttatggatgcctggggtcaaggagcttcagtcactgtctcctca

SEQ ID NO: 129 - DNA, 33 bp, Artificial Sequence
  source: /note="Description of Artificial Sequence: Synthetic oligonucleotide"
aagagtcttctaggtagtaagggcatcaatttc

SEQ ID NO: 130 - DNA, 9 bp, Artificial Sequence
  source: /note="Description of Artificial Sequence: Synthetic oligonucleotide"
cggatgtcc

SEQ ID NO: 131 - DNA, 27 bp, Artificial Sequence
  source: /note="Description of Artificial Sequence: Synthetic oligonucleotide"
gcacagtttctagaatatccgaactcg

SEQ ID NO: 132 - DNA, 396 bp, Artificial Sequence
  source: /note="Description of Artificial Sequence: Synthetic polynucleotide"
atgaagtttcctgctcagtttcttggactgatagtgctctgtattcctggagccactggggatattgtgttgactcaagctccactctctgtttctgtcactcctggagagtcagcttccatctcctgcaggtctagtaagagtcttctaggtagtaagggcatcaatttcttgtattggtaccttcagaagccaggaaagtctcctcagctcctgatatatcggatgtccaaccttgcctcaggagttccagacaggtttagtggtagtgggtcagaaacagattttatactgaagatcagtaaggtggagactgaggatgttggcgtttattactgtgcacagtttctagaatatccgaactcgtttggagctgggaccaagttggaactgaaa

SEQ ID NO: 133 - DNA, 24 bp, Artificial Sequence
  source: /note="Description of Artificial Sequence: Synthetic oligonucleotide"
gggttctcgctaaccaactataac

SEQ ID NO: 134 - DNA, 21 bp, Artificial Sequence
  source: /note="Description of Artificial Sequence: Synthetic oligonucleotide"
atgtggagtggtggaaacaca

SEQ ID NO: 135 - DNA, 39 bp, Artificial Sequence
  source: /note="Description of Artificial Sequence: Synthetic oligonucleotide"
gccagagattctggttacggagagggtcgtcttgattac

SEQ ID NO: 136 - DNA, 414 bp, Artificial Sequence
  source: /note="Description of Artificial Sequence: Synthetic polynucleotide"
atggctgtccgggtactgttgctctgcctggtgacatttccaacctgtgccctgtcccaggtgcagctgatggagtcaggacctggcctggtgcagccctcagagaccctgtccctcacctgcactgtctctgggttctcgctaaccaactataacattcactgggttcgacagcctccagggaaaggtctggagtggatgggactaatgtggagtggtggaaacacagattataattcagctctcaaatcccgactgaccatcagcagggacacctccaagaaccaagttttcttaaaaatgaacagtctgcaaagtgaagacacaaccacttactactgtgccagagattctggttacggagagggtcgtcttgattactggggccaaggcgtcatggtcacagtctcctca

SEQ ID NO: 137 - DNA, 18 bp, Artificial Sequence
  source: /note="Description of Artificial Sequence: Synthetic oligonucleotide"
catagtgttggcacaaat

SEQ ID NO: 138 - DNA, 9 bp, Artificial Sequence
  source: /note="Description of Artificial Sequence: Synthetic oligonucleotide"
tatgtctca

SEQ ID NO: 139 - DNA, 27 bp, Artificial Sequence
  source: /note="Description of Artificial Sequence: Synthetic oligonucleotide"
caacagactcaaagttggcccctcacg

SEQ ID NO: 140 - DNA, 381 bp, Artificial Sequence
  source: /note="Description of Artificial Sequence: Synthetic polynucleotide"
atggtgttcaaatttcagatccttggacttctgcttttctggatttcagcctctagaggggacatcgtgctgactcagtctccaaccaccctgtctgtgactccaggagagacagtcagtctttcctgcagggctagccatagtgttggcacaaatctacactggtatcagcaaaaaccaaatgagtctccaaggcttctcatcaagtatgtctcacagtccaattccgggatcccctccaggttcagtgccagtggatcagggacagattttactctcaacatcaaaaatgtggaatttaatgatgtctcaagttatttttgtcaacagactcaaagttggcccctcacgttcggtgctgggaccaagctggagatcaaa

SEQ ID NO: 141 - DNA, 24 bp, Artificial Sequence
  source: /note="Description of Artificial Sequence: Synthetic oligonucleotide"
ggattcactttcagaaattattac

SEQ ID NO: 142 - DNA, 24 bp, Artificial Sequence
  source: /note="Description of Artificial Sequence: Synthetic oligonucleotide"
actggtactggtggtgatttcact

SEQ ID NO: 143 - DNA, 27 bp, Artificial Sequence
  source: /note="Description of Artificial Sequence: Synthetic oligonucleotide"
gcaagggcctatgggtactttgattac

SEQ ID NO: 144 - DNA, 405 bp, Artificial Sequence
  source: /note="Description of Artificial Sequence: Synthetic polynucleotide"
atggacatcaggctcagtttggctttccttgtccttttcataaaaggtgtccagtgtgaggtgcagctggtggagtctgggggaggcttagtgcagcctggaaggtccatgaaactctcctgttcagcctcaggattcactttcagaaattattacatggcctgggtccgccaggctccaacgaggggtctggagtgggtcgcatccactggtactggtggtgatttcacttactatcgagactccgtgaagggccgattcactatctccagagatactgcagaaaacaccctatacttacaaatggacagtctgaggtctgaggacacggccacttattactgtgcaagggcctatgggtactttgattactggggccaaggagtcaaggtcacagtctcctca

SEQ ID NO: 145 - DNA, 18 bp, Artificial Sequence
  source: /note="Description of Artificial Sequence: Synthetic oligonucleotide"
catagtgttggcacaaat

SEQ ID NO: 146 - DNA, 9 bp, Artificial Sequence
  source: /note="Description of Artificial Sequence: Synthetic oligonucleotide"
tatgtctca

SEQ ID NO: 147 - DNA, 27 bp, Artificial Sequence
  source: /note="Description of Artificial Sequence: Synthetic oligonucleotide"
caacagactcaaagttggcccctcacg

SEQ ID NO: 148 - DNA, 381 bp, Artificial Sequence
  source: /note="Description of Artificial Sequence: Synthetic polynucleotide"
atggtgttcaaatttcagatccttggacttctgcttttctggatttcagcctctagaggggacatcgtgctgactcagtctccaaccaccctgtctgtgactccaggagagacagtcagtctttcctgcagggctagccatagtgttggcacaaatctacactggtatcagcaaaaaacaaatgagtctccaaggcttctcatcaagtatgtctcacagtccaattccgggatcccctccaggttcagtgccagtggatcagggacagattttactctcaacatcaaagatgtggagtttgatgatgtctcaagttatttttgtcaacagactcaaagttggcccctcacgttcggttctgggaccaagctggagatcaaa

SEQ ID NO: 149 - DNA, 24 bp, Artificial Sequence
  source: /note="Description of Artificial Sequence: Synthetic oligonucleotide"
ggattcattttcagaaactattac

SEQ ID NO: 150 - DNA, 24 bp, Artificial Sequence
  source: /note="Description of Artificial Sequence: Synthetic oligonucleotide"
actggtactggtggtgatttcact

SEQ ID NO: 151 - DNA, 27 bp, Artificial Sequence
  source: /note="Description of Artificial Sequence: Synthetic oligonucleotide"
gcaagggcctatgggtactttgattac

SEQ ID NO: 152 - DNA, 405 bp, Artificial Sequence
  source: /note="Description of Artificial Sequence: Synthetic polynucleotide"
atggacatcaggctcagtttggctttccttgtccttttcataaaaggtgtccagtgtgaggtgcagctggtggagtctgggggaggcttagtgcagcctggaaggtccatgaaactctcctgttcagcctcaggattcattttcagaaactattacatggcctgggtccgccaggctccaacgaagggtctggagtgggtcgcatccactggtactggtggtgatttcacttactatcgagactccgtgaagggccgattcactatctccagagatactgcagaaagcaccctatacttacaaatggacagtctgaagtctgaggacacggccacttattactgtgcaagggcctatgggtactttgattactggggccaaggagtcaaggtcacagtctcctca

SEQ ID NO: 153 - DNA, 18 bp, Artificial Sequence
  source: /note="Description of Artificial Sequence: Synthetic oligonucleotide"
cagaatatctacaagtac

SEQ ID NO: 154 - DNA, 9 bp, Artificial Sequence
  source: /note="Description of Artificial Sequence: Synthetic oligonucleotide"
aatataaat

SEQ ID NO: 155 - DNA, 24 bp, Artificial Sequence
  source: /note="Description of Artificial Sequence: Synthetic oligonucleotide"
tatcagtataacagtgggcgggcg

SEQ ID NO: 156 - DNA, 375 bp, Artificial Sequence
  source: /note="Description of Artificial Sequence: Synthetic polynucleotide"
atggctccagtacaacttctagggcttttgctgctctgcctccgagccatgagatgtgacatccagatgacccagtctccttcactcctgtcagcatctgagggagacagagtcactctcagctgcaaagcaagtcagaatatctacaagtacttaaactggtatcagcaaaagcttggagaagctcccaaactcctgatatataatataaataatttgcaaacgggcatcccatcaaggttcagtggcagtggatctggtacagatttcacacttaccatcagcagcctgcagcctgaagacgttgccacatattactgctatcagtataacagtgggcgggcgttcggaggaggcaccaagctggaattgaaa

SEQ ID NO: 157 - DNA, 24 bp, Artificial Sequence
  source: /note="Description of Artificial Sequence: Synthetic oligonucleotide"
ggattcactttcagtgactactgg

SEQ ID NO: 158 - DNA, 30 bp, Artificial Sequence
  source: /note="Description of Artificial Sequence: Synthetic oligonucleotide"
attagaaataaacttaataattatgtaaca

SEQ ID NO: 159 - DNA, 45 bp, Artificial Sequence
  source: /note="Description of Artificial Sequence: Synthetic oligonucleotide"
acaaggatacaacgggttattactacgggggaatactttgattac

SEQ ID NO: 160 - DNA, 429 bp, Artificial Sequence
  source: /note="Description of Artificial Sequence: Synthetic polynucleotide"
atggacttgcgactgacttatgtctttattgttgctattttaaaaggtgtcttgtgtgaggtgaaactggaggaatctgggggaggtttggtgcaacctggaatgtccgtgaaactctcttgtgcaacctctggattcactttcagtgactactggatggagtgggtccgccaggctccagggaaggggctagaatgggtagctgaaattagaaataaacttaataattatgtaacaaattatgggaagcctgtgagaggcagattcaccatctcaagagatgattccaaaagtatagtctacctgcaggtgaacagcataagatctgaagatactggtatttattactgtacaaggatacaacgggttattactacgggggaatactttgattactggggccaaggggtcatggtcacagtctcctca

SEQ ID NO: 161 - protein, 6 aa, Artificial Sequence
  source: /note="Description of Artificial Sequence: Synthetic 6xHis tag"
HHHHHH